European Patent Application EP 4 635 982 A1, published October 22, 2025. Title: NKp46抗体及其用途. Applicant: 合肥天港免疫药物有限公司. Application CN. The sequence listing filed with the application follows.

SEQUENCE LISTING (68 sequences)

SEQ ID NO: 1 - protein, 8 aa, synthetic construct
GYTFTTYW

SEQ ID NO: 2 - protein, 8 aa, synthetic construct
INPGNGGT

SEQ ID NO: 3 - protein, 10 aa, synthetic construct
AIRLRFALDY

SEQ ID NO: 4 - protein, 6 aa, synthetic construct
QDVRNF

SEQ ID NO: 5 - skipped

SEQ ID NO: 6 - protein, 9 aa, synthetic construct
QQGNTLPPT

SEQ ID NO: 7 - protein, 8 aa, synthetic construct
GYTFTSYW

SEQ ID NO: 8 - protein, 8 aa, synthetic construct
VVPGSGRT

SEQ ID NO: 9 - protein, 9 aa, synthetic construct
ARVGGYWDY

SEQ ID NO: 10 - protein, 5 aa, synthetic construct
SSVNY

SEQ ID NO: 11 - skipped

SEQ ID NO: 12 - protein, 9 aa, synthetic construct
QQWSSNPYT

SEQ ID NO: 13 - protein, 8 aa, synthetic construct
GFTFSSYA

SEQ ID NO: 14 - protein, 7 aa, synthetic construct
ISSGGIT

SEQ ID NO: 15 - protein, 8 aa, synthetic construct
VRGFLTSY

SEQ ID NO: 16 - protein, 11 aa, synthetic construct
QSLLNSDGKTY

SEQ ID NO: 17 - skipped

SEQ ID NO: 18 - protein, 8 aa, synthetic construct
WQGTHFWT

SEQ ID NO: 19 - protein, 117 aa, synthetic construct
QVQLVQSGAEVKKPGASVKVSCKASGYTFTTYWMHWVKQAPGQGLEWIGEINPGNGGTNYNEKFKRRATMTVDKSISTAYMELSRLRSDDTAVYYCAIRLRFALDYWGQGTLVTVSS

SEQ ID NO: 20 - protein, 107 aa, synthetic construct
DIQMTQSPSSLSASVGDRVTITCRASQDVRNFLNWFQQKPGKAPKLLIYFTSRLHSGVPSRFSGSGSGTDYTFTISSLQPEDIATYFCQQGNTLPPTFGGGTKLEIK

SEQ ID NO: 21 - protein, 117 aa, synthetic construct
QVQLQQPGAELVRPGASVRLSCKASGYTFTTYWMHWVKLRPGQGFEWIGEINPGNGGTNYNEKFKRKATLTVDKSSSTAYMQLSSLTSEDSAVYYCAIRLRFALDYWGQGTSVTVSS

SEQ ID NO: 22 - protein, 107 aa, synthetic construct
DIQMTQTTSSLSASLGDRVTISCRASQDVRNFLNWFQQKPDGTVKLLIYFTSRLHSGVPSRFSGSGSGTDYSLTISNLEQEDIATYFCQQGNTLPPTFGGGTKLEIK

SEQ ID NO: 23 - protein, 116 aa, synthetic construct
QVQLQQSGDDLVKPGASVKLSCKASGYTFTSYWINWIKQRPGQGLEWIGRVVPGSGRTYYNEIFKGKAILTVDSYSNTAYIQLRSVSSEDSAVYFCARVGGYWDYWGQGITLTVSS

SEQ ID NO: 24 - protein, 106 aa, synthetic construct
QIVLSQSPAILSASPGEKVTMACRASSSVNYIHWYQQRPGSSPKPWIYATSSLASGVPARFSGSGSGTSYSLTISRVEAEDAATYYCQQWSSNPYTFGGGTKLEMK

SEQ ID NO: 25 - protein, 114 aa, synthetic construct
EVKLVESGGGLVKPGGSLKLSCAPFGFTFSSYAMSWVRQTPEKRLEWVASISSGGITYYPDSVKGRFTISRDNVRNILNLQMSSLRSEDTAMYYCVRGFLTSYWGQGTLVTVSA

SEQ ID NO: 26 - protein, 111 aa, synthetic construct
DVVMTQTPLTLSVTIGQPASISCKSSQSLLNSDGKTYLNWLLQRPGQSPKRLISLVSKLDSGVPDRFTGSGSGTDFTLKISRVEAEDLGVYYCWQGTHFWTFGGGTKLEIK

SEQ ID NO: 27 - protein, 330 aa, synthetic construct
ASTKGPSVFPLAPSSKSTSGGTAALGCLVKDYFPEPVTVSWNSGALTSGVHTFPAVLQSSGLYSLSSVVTVPSSSLGTQTYICNVNHKPSNTKVDKKVEPKSCDKTHTCPPCPAPEAAGGPSVFLFPPKPKDTLMISRTPEVTCVVVDVSHEDPEVKFNWYVDGVEVHNAKTKPREEQYNSTYRVVSVLTVLHQDWLNGKEYKCKVSNKALPAPIEKTISKAKGQPREPQVYTLPPSREEMTKNQVSLTCLVKGFYPSDIAVEWESNGQPENNYKTTPPVLDSDGSFFLYSKLTVDKSRWQQGNVFSCSVMHEALHNHYTQKSLSLSPGK

SEQ ID NO: 28 - protein, 330 aa, synthetic construct
AKTTAPSVYPLAPVCGDTTGSSVTLGCLVKGYFPEPVTLTWNSGSLSSGVHTFPAVLQSDLYTLSSSVTVTSSTWPSQSITCNVAHPASSTKVDKKIEPRGPTIKPCPPCKCPAPNLLGGPSVFIFPPKIKDVLMISLSPIVTCVVVDVSEDDPDVQISWFVNNVEVHTAQTQTHREDYNSTLRVVSALPIQHQDWMSGKEFKCKVNNKDLPAPIERTISKPKGSVRAPQVYVLPPPEEEMTKKQVTLTCMVTDFMPEDIYVEWTNNGKTELNYKNTEPVLDSDGSYFMYSKLRVEKKNWVERNSYSCSVVHEGLHNHHTTKSFSRTPGK

SEQ ID NO: 29 - protein, 447 aa, synthetic construct
QVQLVQSGAEVKKPGASVKVSCKASGYTFTTYWMHWVKQAPGQGLEWIGEINPGNGGTNYNEKFKRRATMTVDKSISTAYMELSRLRSDDTAVYYCAIRLRFALDYWGQGTLVTVSSASTKGPSVFPLAPSSKSTSGGTAALGCLVKDYFPEPVTVSWNSGALTSGVHTFPAVLQSSGLYSLSSVVTVPSSSLGTQTYICNVNHKPSNTKVDKKVEPKSCDKTHTCPPCPAPEAAGGPSVFLFPPKPKDTLMISRTPEVTCVVVDVSHEDPEVKFNWYVDGVEVHNAKTKPREEQYNSTYRVVSVLTVLHQDWLNGKEYKCKVSNKALPAPIEKTISKAKGQPREPQVYTLPPSREEMTKNQVSLTCLVKGFYPSDIAVEWESNGQPENNYKTTPPVLDSDGSFFLYSKLTVDKSRWQQGNVFSCSVMHEALHNHYTQKSLSLSPGK

SEQ ID NO: 30 - protein, 214 aa, synthetic construct
DIQMTQSPSSLSASVGDRVTITCRASQDVRNFLNWFQQKPGKAPKLLIYFTSRLHSGVPSRFSGSGSGTDYTFTISSLQPEDIATYFCQQGNTLPPTFGGGTKLEIKRTVAAPSVFIFPPSDEQLKSGTASVVCLLNNFYPREAKVQWKVDNALQSGNSQESVTEQDSKDSTYSLSSTLTLSKADYEKHKVYACEVTHQGLSSPVTKSFNRGEC

SEQ ID NO: 31 - protein, 447 aa, synthetic construct
QVQLQQPGAELVRPGASVRLSCKASGYTFTTYWMHWVKLRPGQGFEWIGEINPGNGGTNYNEKFKRKATLTVDKSSSTAYMQLSSLTSEDSAVYYCAIRLRFALDYWGQGTSVTVSSASTKGPSVFPLAPSSKSTSGGTAALGCLVKDYFPEPVTVSWNSGALTSGVHTFPAVLQSSGLYSLSSVVTVPSSSLGTQTYICNVNHKPSNTKVDKKVEPKSCDKTHTCPPCPAPEAAGGPSVFLFPPKPKDTLMISRTPEVTCVVVDVSHEDPEVKFNWYVDGVEVHNAKTKPREEQYNSTYRVVSVLTVLHQDWLNGKEYKCKVSNKALPAPIEKTISKAKGQPREPQVYTLPPSREEMTKNQVSLTCLVKGFYPSDIAVEWESNGQPENNYKTTPPVLDSDGSFFLYSKLTVDKSRWQQGNVFSCSVMHEALHNHYTQKSLSLSPGK

SEQ ID NO: 32 - protein, 214 aa, synthetic construct
DIQMTQTTSSLSASLGDRVTISCRASQDVRNFLNWFQQKPDGTVKLLIYFTSRLHSGVPSRFSGSGSGTDYSLTISNLEQEDIATYFCQQGNTLPPTFGGGTKLEIKRTVAAPSVFIFPPSDEQLKSGTASVVCLLNNFYPREAKVQWKVDNALQSGNSQESVTEQDSKDSTYSLSSTLTLSKADYEKHKVYACEVTHQGLSSPVTKSFNRGEC

SEQ ID NO: 33 - protein, 447 aa, synthetic construct
QVQLQQPGAELVRPGASVRLSCKASGYTFTTYWMHWVKLRPGQGFEWIGEINPGNGGTNYNEKFKRKATLTVDKSSSTAYMQLSSLTSEDSAVYYCAIRLRFALDYWGQGTSVTVSSAKTTAPSVYPLAPVCGDTTGSSVTLGCLVKGYFPEPVTLTWNSGSLSSGVHTFPAVLQSDLYTLSSSVTVTSSTWPSQSITCNVAHPASSTKVDKKIEPRGPTIKPCPPCKCPAPNLLGGPSVFIFPPKIKDVLMISLSPIVTCVVVDVSEDDPDVQISWFVNNVEVHTAQTQTHREDYNSTLRVVSALPIQHQDWMSGKEFKCKVNNKDLPAPIERTISKPKGSVRAPQVYVLPPPEEEMTKKQVTLTCMVTDFMPEDIYVEWTNNGKTELNYKNTEPVLDSDGSYFMYSKLRVEKKNWVERNSYSCSVVHEGLHNHHTTKSFSRTPGK

SEQ ID NO: 34 - protein, 214 aa, synthetic construct
DIQMTQTTSSLSASLGDRVTISCRASQDVRNFLNWFQQKPDGTVKLLIYFTSRLHSGVPSRFSGSGSGTDYSLTISNLEQEDIATYFCQQGNTLPPTFGGGTKLEIKRADAAPTVSIFPPSSEQLTSGGASVVCFLNNFYPKDINVKWKIDGSERQNGVLNSWTDQDSKDSTYSMSSTLTLTKDEYERHNSYTCEATHKTSTSPIVKSFNRNEC

SEQ ID NO: 35 - protein, 446 aa, synthetic construct
QVQLQQSGDDLVKPGASVKLSCKASGYTFTSYWINWIKQRPGQGLEWIGRVVPGSGRTYYNEIFKGKAILTVDSYSNTAYIQLRSVSSEDSAVYFCARVGGYWDYWGQGITLTVSSASTKGPSVFPLAPSSKSTSGGTAALGCLVKDYFPEPVTVSWNSGALTSGVHTFPAVLQSSGLYSLSSVVTVPSSSLGTQTYICNVNHKPSNTKVDKKVEPKSCDKTHTCPPCPAPEAAGGPSVFLFPPKPKDTLMISRTPEVTCVVVDVSHEDPEVKFNWYVDGVEVHNAKTKPREEQYNSTYRVVSVLTVLHQDWLNGKEYKCKVSNKALPAPIEKTISKAKGQPREPQVYTLPPSREEMTKNQVSLTCLVKGFYPSDIAVEWESNGQPENNYKTTPPVLDSDGSFFLYSKLTVDKSRWQQGNVFSCSVMHEALHNHYTQKSLSLSPGK

SEQ ID NO: 36 - protein, 213 aa, synthetic construct
QIVLSQSPAILSASPGEKVTMACRASSSVNYIHWYQQRPGSSPKPWIYATSSLASGVPARFSGSGSGTSYSLTISRVEAEDAATYYCQQWSSNPYTFGGGTKLEMKRTVAAPSVFIFPPSDEQLKSGTASVVCLLNNFYPREAKVQWKVDNALQSGNSQESVTEQDSKDSTYSLSSTLTLSKADYEKHKVYACEVTHQGLSSPVTKSFNRGEC

SEQ ID NO: 37 - protein, 446 aa, synthetic construct
QVQLQQSGDDLVKPGASVKLSCKASGYTFTSYWINWIKQRPGQGLEWIGRVVPGSGRTYYNEIFKGKAILTVDSYSNTAYIQLRSVSSEDSAVYFCARVGGYWDYWGQGITLTVSSAKTTAPSVYPLAPVCGDTTGSSVTLGCLVKGYFPEPVTLTWNSGSLSSGVHTFPAVLQSDLYTLSSSVTVTSSTWPSQSITCNVAHPASSTKVDKKIEPRGPTIKPCPPCKCPAPNLLGGPSVFIFPPKIKDVLMISLSPIVTCVVVDVSEDDPDVQISWFVNNVEVHTAQTQTHREDYNSTLRVVSALPIQHQDWMSGKEFKCKVNNKDLPAPIERTISKPKGSVRAPQVYVLPPPEEEMTKKQVTLTCMVTDFMPEDIYVEWTNNGKTELNYKNTEPVLDSDGSYFMYSKLRVEKKNWVERNSYSCSVVHEGLHNHHTTKSFSRTPGK

SEQ ID NO: 38 - protein, 213 aa, synthetic construct
QIVLSQSPAILSASPGEKVTMACRASSSVNYIHWYQQRPGSSPKPWIYATSSLASGVPARFSGSGSGTSYSLTISRVEAEDAATYYCQQWSSNPYTFGGGTKLEMKRADAAPTVSIFPPSSEQLTSGGASVVCFLNNFYPKDINVKWKIDGSERQNGVLNSWTDQDSKDSTYSMSSTLTLTKDEYERHNSYTCEATHKTSTSPIVKSFNRNEC

SEQ ID NO: 39 - protein, 444 aa, synthetic construct
EVKLVESGGGLVKPGGSLKLSCAPFGFTFSSYAMSWVRQTPEKRLEWVASISSGGITYYPDSVKGRFTISRDNVRNILNLQMSSLRSEDTAMYYCVRGFLTSYWGQGTLVTVSAASTKGPSVFPLAPSSKSTSGGTAALGCLVKDYFPEPVTVSWNSGALTSGVHTFPAVLQSSGLYSLSSVVTVPSSSLGTQTYICNVNHKPSNTKVDKKVEPKSCDKTHTCPPCPAPEAAGGPSVFLFPPKPKDTLMISRTPEVTCVVVDVSHEDPEVKFNWYVDGVEVHNAKTKPREEQYNSTYRVVSVLTVLHQDWLNGKEYKCKVSNKALPAPIEKTISKAKGQPREPQVYTLPPSREEMTKNQVSLTCLVKGFYPSDIAVEWESNGQPENNYKTTPPVLDSDGSFFLYSKLTVDKSRWQQGNVFSCSVMHEALHNHYTQKSLSLSPGK

SEQ ID NO: 40 - protein, 218 aa, synthetic construct
DVVMTQTPLTLSVTIGQPASISCKSSQSLLNSDGKTYLNWLLQRPGQSPKRLISLVSKLDSGVPDRFTGSGSGTDFTLKISRVEAEDLGVYYCWQGTHFWTFGGGTKLEIKRTVAAPSVFIFPPSDEQLKSGTASVVCLLNNFYPREAKVQWKVDNALQSGNSQESVTEQDSKDSTYSLSSTLTLSKADYEKHKVYACEVTHQGLSSPVTKSFNRGEC

SEQ ID NO: 41 - protein, 444 aa, synthetic construct
EVKLVESGGGLVKPGGSLKLSCAPFGFTFSSYAMSWVRQTPEKRLEWVASISSGGITYYPDSVKGRFTISRDNVRNILNLQMSSLRSEDTAMYYCVRGFLTSYWGQGTLVTVSAAKTTAPSVYPLAPVCGDTTGSSVTLGCLVKGYFPEPVTLTWNSGSLSSGVHTFPAVLQSDLYTLSSSVTVTSSTWPSQSITCNVAHPASSTKVDKKIEPRGPTIKPCPPCKCPAPNLLGGPSVFIFPPKIKDVLMISLSPIVTCVVVDVSEDDPDVQISWFVNNVEVHTAQTQTHREDYNSTLRVVSALPIQHQDWMSGKEFKCKVNNKDLPAPIERTISKPKGSVRAPQVYVLPPPEEEMTKKQVTLTCMVTDFMPEDIYVEWTNNGKTELNYKNTEPVLDSDGSYFMYSKLRVEKKNWVERNSYSCSVVHEGLHNHHTTKSFSRTPGK

SEQ ID NO: 42 - protein, 218 aa, synthetic construct
DVVMTQTPLTLSVTIGQPASISCKSSQSLLNSDGKTYLNWLLQRPGQSPKRLISLVSKLDSGVPDRFTGSGSGTDFTLKISRVEAEDLGVYYCWQGTHFWTFGGGTKLEIKRADAAPTVSIFPPSSEQLTSGGASVVCFLNNFYPKDINVKWKIDGSERQNGVLNSWTDQDSKDSTYSMSSTLTLTKDEYERHNSYTCEATHKTSTSPIVKSFNRNEC

SEQ ID NO: 43 - protein, 231 aa, synthetic construct
PKSSDKTHTCPPCPAPEAAGGPSVFLFPPKPKDTLMISRTPEVTCVVVDVSHEDPEVKFNWYVDGVEVHNAKTKPREEQYNSTYRVVSVLTVLHQDWLNGKEYKCKVSNKALPAPIEKTISKAKGQPREPQVYTLPPCREEMTKNQVSLWCLVKGFYPSDIAVEWESNGQPENNYKTTPPVLDSDGSFFLYSKLTVDKSRWQQGNVFSCSVMHEALHNHYTQKSLSLSPGK

SEQ ID NO: 44 - protein, 15 aa, synthetic construct
GGGGSGGGGSGGGGS

SEQ ID NO: 45 - protein, 239 aa, synthetic construct
QVQLQQPGAELVRPGASVRLSCKASGYTFTTYWMHWVKLRPGQGFEWIGEINPGNGGTNYNEKFKRKATLTVDKSSSTAYMQLSSLTSEDSAVYYCAIRLRFALDYWGQGTSVTVSSGGGGSGGGGSGGGGSDIQMTQTTSSLSASLGDRVTISCRASQDVRNFLNWFQQKPDGTVKLLIYFTSRLHSGVPSRFSGSGSGTDYSLTISNLEQEDIATYFCQQGNTLPPTFGGGTKLEIK

SEQ ID NO: 46 - protein, 475 aa, synthetic construct
QVQLVQSGAEVKKPGASVKVSCKASGYTFTTYWMHWVKQAPGQGLEWIGEINPGNGGTNYNEKFKRRATMTVDKSISTAYMELSRLRSDDTAVYYCAIRLRFALDYWGQGTLVTVSSGGGGSGGGGSGGGGSDIQMTQSPSSLSASVGDRVTITCRASQDVRNFLNWFQQKPGKAPKLLIYFTSRLHSGVPSRFSGSGSGTDYTFTISSLQPEDIATYFCQQGNTLPPTFGGGTKLEIKGGGGSPKSSDKTHTCPPCPAPEAAGGPSVFLFPPKPKDTLMISRTPEVTCVVVDVSHEDPEVKFNWYVDGVEVHNAKTKPREEQYNSTYRVVSVLTVLHQDWLNGKEYKCKVSNKALPAPIEKTISKAKGQPREPQVYTLPPCREEMTKNQVSLWCLVKGFYPSDIAVEWESNGQPENNYKTTPPVLDSDGSFFLYSKLTVDKSRWQQGNVFSCSVMHEALHNHYTQKSLSLSPGK

SEQ ID NO: 47 - protein, 239 aa, synthetic construct; identical to SEQ ID NO: 45

SEQ ID NO: 48 - protein, 475 aa, synthetic construct
QVQLQQPGAELVRPGASVRLSCKASGYTFTTYWMHWVKLRPGQGFEWIGEINPGNGGTNYNEKFKRKATLTVDKSSSTAYMQLSSLTSEDSAVYYCAIRLRFALDYWGQGTSVTVSSGGGGSGGGGSGGGGSDIQMTQTTSSLSASLGDRVTISCRASQDVRNFLNWFQQKPDGTVKLLIYFTSRLHSGVPSRFSGSGSGTDYSLTISNLEQEDIATYFCQQGNTLPPTFGGGTKLEIKGGGGSPKSSDKTHTCPPCPAPEAAGGPSVFLFPPKPKDTLMISRTPEVTCVVVDVSHEDPEVKFNWYVDGVEVHNAKTKPREEQYNSTYRVVSVLTVLHQDWLNGKEYKCKVSNKALPAPIEKTISKAKGQPREPQVYTLPPCREEMTKNQVSLWCLVKGFYPSDIAVEWESNGQPENNYKTTPPVLDSDGSFFLYSKLTVDKSRWQQGNVFSCSVMHEALHNHYTQKSLSLSPGK

SEQ ID NO: 49 - protein, 231 aa, synthetic construct
PKSCDKTHTCPPCPAPEAAGGPSVFLFPPKPKDTLMISRTPEVTCVVVDVSHEDPEVKFNWYVDGVEVHNAKTKPREEQYNSTYRVVSVLTVLHQDWLNGKEYKCKVSNKALPAPIEKTISKAKGQPREPQVCTLPPSREEMTKNQVSLSCAVKGFYPSDIAVEWESNGQPENNYKTTPPVLDSDGSFFLVSKLTVDKSRWQQGNVFSCSVMHEALHNHYTQKSLSLSPGK

SEQ ID NO: 50 - protein, 231 aa, synthetic construct
PKSCDKTHTCPPCPAPELLGGPSVFLFPPKPKDTLMISRTPEVTCVVVDVSHEDPEVKFNWYVDGVEVHNAKTKPREEQYNSTYRVVSVLTVLHQDWLNGKEYKCKVSNKALPAPIEKTISKAKGQPREPQVYTLPPSREEMTKNQVSLTCLVKGFYPSDIAVEWESNGQPENNYKTTPPVLDSDGSFFLYSKLTVDKSRWQQGNVFSCSVMHEALHNHYTQKSLSLSPGK

SEQ ID NO: 51 - protein, 119 aa, synthetic construct
QVQLQESGPGLVKPSETLSLTCTVSGFSLTTYGVHWIRQPPGKGLEWIGMIWTDATTDYNAAFISRVTISVDTSKNQFSLKLSSVTAADTAVYYCARKGHGYYYAMDYWGQGTLVTVSS

SEQ ID NO: 52 - protein, 108 aa, synthetic construct
EIVLTQSPGTLSLSPGERATLSCTASSSVSSSYLHWYQQKPGQAPRLLIYSTSNLASGIPDRFSGSGSGTDFTLTISRLEPEDFAVYYCHQYHRSPFTFGQGTKLEIK

SEQ ID NO: 53 - protein, 449 aa, synthetic construct
QVQLQESGPGLVKPSETLSLTCTVSGFSLTTYGVHWIRQPPGKGLEWIGMIWTDATTDYNAAFISRVTISVDTSKNQFSLKLSSVTAADTAVYYCARKGHGYYYAMDYWGQGTLVTVSSASTKGPSVFPLAPSSKSTSGGTAALGCLVKDYFPEPVTVSWNSGALTSGVHTFPAVLQSSGLYSLSSVVTVPSSSLGTQTYICNVNHKPSNTKVDKKVEPKSCDKTHTCPPCPAPEAAGGPSVFLFPPKPKDTLMISRTPEVTCVVVDVSHEDPEVKFNWYVDGVEVHNAKTKPREEQYNSTYRVVSVLTVLHQDWLNGKEYKCKVSNKALPAPIEKTISKAKGQPREPQVCTLPPSREEMTKNQVSLSCAVKGFYPSDIAVEWESNGQPENNYKTTPPVLDSDGSFFLVSKLTVDKSRWQQGNVFSCSVMHEALHNHYTQKSLSLSPGK

SEQ ID NO: 54 - protein, 215 aa, synthetic construct
EIVLTQSPGTLSLSPGERATLSCTASSSVSSSYLHWYQQKPGQAPRLLIYSTSNLASGIPDRFSGSGSGTDFTLTISRLEPEDFAVYYCHQYHRSPFTFGQGTKLEIKRTVAAPSVFIFPPSDEQLKSGTASVVCLLNNFYPREAKVQWKVDNALQSGNSQESVTEQDSKDSTYSLSSTLTLSKADYEKHKVYACEVTHQGLSSPVTKSFNRGEC

SEQ ID NO: 55 - protein, 107 aa, synthetic construct [sequence omitted]

SEQ ID NO: 56 - protein, 107 aa, synthetic construct
RADAAPTVSIFPPSSEQLTSGGASVVCFLNNFYPKDINVKWKIDGSERQNGVLNSWTDQDSKDSTYSMSSTLTLTKDEYERHNSYTCEATHKTSTSPIVKSFNRNEC

SEQ ID NO: 57 - protein, 237 aa, synthetic construct
QVQLQQSGDDLVKPGASVKLSCKASGYTFTSYWINWIKQRPGQGLEWIGRVVPGSGRTYYNEIFKGKAILTVDSYSNTAYIQLRSVSSEDSAVYFCARVGGYWDYWGQGITLTVSSGGGGSGGGGSGGGGSQIVLSQSPAILSASPGEKVTMACRASSSVNYIHWYQQRPGSSPKPWIYATSSLASGVPARFSGSGSGTSYSLTISRVEAEDAATYYCQQWSSNPYTFGGGTKLEMK

SEQ ID NO: 58 - protein, 473 aa, synthetic construct
QVQLQQSGDDLVKPGASVKLSCKASGYTFTSYWINWIKQRPGQGLEWIGRVVPGSGRTYYNEIFKGKAILTVDSYSNTAYIQLRSVSSEDSAVYFCARVGGYWDYWGQGITLTVSSGGGGSGGGGSGGGGSQIVLSQSPAILSASPGEKVTMACRASSSVNYIHWYQQRPGSSPKPWIYATSSLASGVPARFSGSGSGTSYSLTISRVEAEDAATYYCQQWSSNPYTFGGGTKLEMKGGGGSPKSSDKTHTCPPCPAPEAAGGPSVFLFPPKPKDTLMISRTPEVTCVVVDVSHEDPEVKFNWYVDGVEVHNAKTKPREEQYNSTYRVVSVLTVLHQDWLNGKEYKCKVSNKALPAPIEKTISKAKGQPREPQVYTLPPCREEMTKNQVSLWCLVKGFYPSDIAVEWESNGQPENNYKTTPPVLDSDGSFFLYSKLTVDKSRWQQGNVFSCSVMHEALHNHYTQKSLSLSPGK

SEQ ID NO: 59 - protein, 240 aa, synthetic construct
EVKLVESGGGLVKPGGSLKLSCAPFGFTFSSYAMSWVRQTPEKRLEWVASISSGGITYYPDSVKGRFTISRDNVRNILNLQMSSLRSEDTAMYYCVRGFLTSYWGQGTLVTVSAGGGGSGGGGSGGGGSDVVMTQTPLTLSVTIGQPASISCKSSQSLLNSDGKTYLNWLLQRPGQSPKRLISLVSKLDSGVPDRFTGSGSGTDFTLKISRVEAEDLGVYYCWQGTHFWTFGGGTKLEIK

SEQ ID NO: 60 - protein, 476 aa, synthetic construct
EVKLVESGGGLVKPGGSLKLSCAPFGFTFSSYAMSWVRQTPEKRLEWVASISSGGITYYPDSVKGRFTISRDNVRNILNLQMSSLRSEDTAMYYCVRGFLTSYWGQGTLVTVSAGGGGSGGGGSGGGGSDVVMTQTPLTLSVTIGQPASISCKSSQSLLNSDGKTYLNWLLQRPGQSPKRLISLVSKLDSGVPDRFTGSGSGTDFTLKISRVEAEDLGVYYCWQGTHFWTFGGGTKLEIKGGGGSPKSSDKTHTCPPCPAPEAAGGPSVFLFPPKPKDTLMISRTPEVTCVVVDVSHEDPEVKFNWYVDGVEVHNAKTKPREEQYNSTYRVVSVLTVLHQDWLNGKEYKCKVSNKALPAPIEKTISKAKGQPREPQVYTLPPCREEMTKNQVSLWCLVKGFYPSDIAVEWESNGQPENNYKTTPPVLDSDGSFFLYSKLTVDKSRWQQGNVFSCSVMHEALHNHYTQKSLSLSPGK

SEQ ID NO: 61 - protein, 304 aa, synthetic construct
MSSTLPALLCVGLCLSQRISAQQQTLPKPFIWAEPHFMVPKEKQVTICCQGNYGAVEYQLHFEGSLFAVDRPKPPERINKVKFYIPDMNSRMAGQYSCIYRVGELWSEPSNLLDLVVTEMYDTPTLSVHPGPEVISGEKVTFYCRLDTATSMFLLLKEGRSSHVQRGYGKVQAEFPLGPVTTAHRGTYRCFGSYNNHAWSFPSEPVKLLVTGDIENTSLAPEDPTFPADTWGTYLLTTETGLQKDHALWDHTAQNLLRMGLAFLVLVALVWFLVEDWLSRKRTRERASRASTWEGRRRLNTQTL

SEQ ID NO: 62 - protein, 445 aa, synthetic construct
QVQLQQPGSELVRPGASVKLSCKASGYTFTSYWMHWVKQRPGQGLEWIGTIYPGSDITNYDEKFKNKATLTVDTSSSTAYMQLSSLTSEDSAVYYCTRDGRFANWGQGTLVTVSAASTKGPSVFPLAPSSKSTSGGTAALGCLVKDYFPEPVTVSWNSGALTSGVHTFPAVLQSSGLYSLSSVVTVPSSSLGTQTYICNVNHKPSNTKVDKKVEPKSCDKTHTCPPCPAPEAAGGPSVFLFPPKPKDTLMISRTPEVTCVVVDVSHEDPEVKFNWYVDGVEVHNAKTKPREEQYNSTYRVVSVLTVLHQDWLNGKEYKCKVSNKALPAPIEKTISKAKGQPREPQVYTLPPSREEMTKNQVSLTCLVKGFYPSDIAVEWESNGQPENNYKTTPPVLDSDGSFFLYSKLTVDKSRWQQGNVFSCSVMHEALHNHYTQKSLSLSPGK

SEQ ID NO: 63 - protein, 214 aa, synthetic construct
EIQMTQSPSSLSASLGERVSLTCRASQDIGSSLNWLQQEPDGTIKRLIYATSSLDSGVPKRFSGSRSGSDYSLTISSLESEDFVDYYCLQYASSPYTFGGGTKLEIKRTVAAPSVFIFPPSDEQLKSGTASVVCLLNNFYPREAKVQWKVDNALQSGNSQESVTEQDSKDSTYSLSSTLTLSKADYEKHKVYACEVTHQGLSSPVTKSFNRGEC

SEQ ID NO: 64 - protein, 453 aa, synthetic construct
QVTLKESGPGILQPSQTLSLTCSFSGFSLSTYGIGVGWNRQPSGKGLEWLAHIWWNDNEYYNIDLKSRLTISKDTSNNQVFLKIASVDTADTATYYCVRGNYRYARGYVMDYWGQGTSVTVSSASTKGPSVFPLAPSSKSTSGGTAALGCLVKDYFPEPVTVSWNSGALTSGVHTFPAVLQSSGLYSLSSVVTVPSSSLGTQTYICNVNHKPSNTKVDKKVEPKSCDKTHTCPPCPAPEAAGGPSVFLFPPKPKDTLMISRTPEVTCVVVDVSHEDPEVKFNWYVDGVEVHNAKTKPREEQYNSTYRVVSVLTVLHQDWLNGKEYKCKVSNKALPAPIEKTISKAKGQPREPQVYTLPPSREEMTKNQVSLTCLVKGFYPSDIAVEWESNGQPENNYKTTPPVLDSDGSFFLYSKLTVDKSRWQQGNVFSCSVMHEALHNHYTQKSLSLSPGK

SEQ ID NO: 65 - protein, 218 aa, synthetic construct
DIVLTQSPASLAVSLGQRATISCRASESVEYYGTSLMQWYQQKPGQPPKLLIYAASNVESGVPARFSGSGSGTDFSLNIHPVEEDDFAMYFCQQNRKVPWTFGGGTKLEIKRTVAAPSVFIFPPSDEQLKSGTASVVCLLNNFYPREAKVQWKVDNALQSGNSQESVTEQDSKDSTYSLSSTLTLSKADYEKHKVYACEVTHQGLSSPVTKSFNRGEC

SEQ ID NO: 66 - protein, 99 aa, synthetic construct
ASTKGPSVFPLAPSSKSTSGGTAALGCLVKDYFPEPVTVSWNSGALTSGVHTFPAVLQSSGLYSLSSVVTVPSSSLGTQTYICNVNHKPSNTKVDKKVE

SEQ ID NO: 67 - protein, 107 aa, synthetic construct [sequence omitted]

SEQ ID NO: 68 - protein, 5 aa, synthetic construct
GGGGS